European Patent Specification EP 3 865 212 B1, published March 13, 2024. Title: MICROFLUIDIC DEVICES AND METHODS FOR USE THEREOF IN MULTICELLULAR ASSAYS OF SECRETION. Applicant: THE UNIVERSITY OF BRITISH COLUMBIA. The sequence listing filed with the application follows.

SEQUENCE LISTING (85 sequences)

SEQ ID NO: 1 - DNA, 395 bp, Mus sp.
atggaatggacctgggtctttctcttcctcctgtcagtaactgcaggtgtccactcccaggttcagctgcagcagtctggacctgagctgatgaagcctggggcctcagtgaagatatcctgcaaggcaactggctacacattcagaaactactggatagagtggataaagcagaggcctggacatggccttgagtggattggagagattttacctgaaagtggtagtattaattacaatgagaaattcaagggcaaggccacattcactgcagatacatcctccaacacagcctacttgcaactccgcagcctgacatctgaggactctgccgtctattattgtttttatgataattacgtttttgactactggggccaaggcaccactctcac

SEQ ID NO: 2 - protein, 131 aa, Mus sp.
MEWTWVFLFLLSVTAGVHSQVQLQQSGPELMKPGASVKISCKATGYTFRNYWIEWIKQRPGHGLEWIGEILPESGSINYNEKFKGKATFTADTSSNTAYLQLRSLTSEDSAVYYCFYDNYVFDYWGQGTTL

SEQ ID NO: 3 - DNA, 372 bp, Mus sp.
atggattctcaagtgcagattttcagcttcctgctaatcagtgcctcggtcatactatccagtggacaaattgttctcatccagtctccaacaatcatgtctgcatctccaggggagaaggtcaccatgacctgcagtgccaactcaagtttcagttacatgcactggtaccagcagaagtcaggcacctcccccaaaagatggatttatgacacatccaaactggcttctggagtccctgctcgcttcagtggcagtgggtctgggacctcttactctctcacaattagcagcatggaggctgaagatgctgccacttattactgtcagcagtggagtagaaaccccacgttcggtgctggaccaagctga

SEQ ID NO: 4 - protein, 124 aa, Mus sp.
MDSQVQIFSFLLISASVILSSGQIVLIQSPTIMSASPGEKVTMTCSANSSFSYMHWYQQKSGTSPKRWIYDTSKLASGVPARFSGSGSGTSYSLTISSMEAEDAATYYCQQWSRNPTFGAGTKL

SEQ ID NO: 5 - DNA, 347 bp, Mus sp.
atgcaagcagtggtatcaacgcagagtacggggaaggagtcaggacctggcttggtggcgccctcacagagcatgtccatcatgtgcactgtctctgggttttcattaagcaactatggtgtacactgggttcgccagcctccaggaaagggtctggagtggctgggagtaatttgggctggtggaaacacaaattataattcggctctcatgtccagactgagcatcagcaaagacaagtccaagagtcaagttttcttaaaaatgaaccgtctggaaactgatgacacagccatgtactatctgtgccagtgtaggatggttaccccttgcttactgggccaagg

SEQ ID NO: 6 - protein, 115 aa, Mus sp.
MQAVVSTQSTGKESGPGLVAPSQSMSIMCTVSGFSLSNYGVHWVRQPPGKGLEWLGVIWAGGNTNYNSALMSRLSISKDKSKSQVFLKMNRLETDDTAMYYLCQCRMVTPCLLGQ

SEQ ID NO: 7 - DNA, 369 bp, Mus sp.
atggagtcacagattcaggtctttgtattcgtgtttctctggttgtctggtgttgacggagacattgtgatgacccagtctcacaaattcatgtccacatcagtaggagacagggtcagcatcacctgcaaggccagtcaggatgtgagtatttctgtagcctggtatcaacagaaaccaggacaatctcctaaactactgatttactcggcatcctaccggtacactggagtccctgatcgcttcactggcagtggatctgggacggatttcactttcaccatccgcagtgtgcaggctgaagacctggcagtttattactgtcagcaacattatagtactcctttcacgtcggctcgggacaaagtg

SEQ ID NO: 8 - protein, 123 aa, Mus sp.
MESQIQVFVFVFLWLSGVDGDIVMTQSHKFMSTSVGDRVSITCKASQDVSISVAWYQQKPGQSPKLLIYSASYRYTGVPDRFTGSGSGTDFTFTIRSVQAEDLAVYYCQQHYSTPFTSARDKV

SEQ ID NO: 9 - DNA, 545 bp, Homo sapiens
atgaagcacctgtggttcttcctcctgctggtggcggctcccagatgggtcctgtctcaggtgcagctgcaggagtcgggcccaggactggtgaagtcttcggagaccctgtccctcacctgcactgtctctggtgactccatcaccagcagtacttacgactggggctggatccgtcagccccccgggaagggcctggagtggattggcaatgtctattatagagggagcacctactacaacccgtccctcaagagtcgagtcaccatatccgtagacaggtccaggacccagatctccctgaggctgagctctgtgaccgccgctgacacggctctgtatttctgtgcgagacacccgaaacgtctaacggtttttgaagtggtcaacgcttttgatatctggggccaagggacaatggtcaccgtcttttcagcctccaccaagggcccatcggtcttccccctggcaccctcctccaagagcacctctgggggcacagcggccctgggctgcctggtctgctgacgaggcactgaggactg

SEQ ID NO: 10 - protein, 169 aa, Homo sapiens
MKHLWFFLLLVAAPRWVLSQVQLQESGPGLVKSSETLSLTCTVSGDSITSSTYDWGWIRQPPGKGLEWIGNVYYRGSTYYNPSLKSRVTISVDRSRTQISLRLSSVTAADTALYFCARHPKRLTVFEVVNAFDIWGQGQTMVTVFSASTKGPSVFPLAPSSKSTSGGTA

SEQ ID NO: 11 - DNA, 465 bp, Homo sapiens
atggcctgggctctgctactcctcaccctcctcactcagggcacagggtcctgggcccagtctgccctgactcagcctgcctccgtgtctgcatctcctggacagtcgatcaccatctcctgcactggaatcagcagtgacattggtggttatagctctgtctcctggtaccaagcgcacccaggcaaagcccccaaactcatgatctatgatgtcaataatcggccctcaggcatttctaatcgcttctctggttccaagtctggcaacacggcctccctggccatctctgggctccaggctgaggacgaggcagattattactgcagcttatatacaagtatcaacgcttccatagtgttcggcggagggaccaagctgaccgtcctaggtcagcccaaggctgccccctcggtcactctgttcccgccctcctctgaggagcttcaagccaacaaggccaca

SEQ ID NO: 12 - protein, 146 aa, Homo sapiens
MAWALLLLTLLTQGTGSWAQSALTQPASVSASPGQSITISCTGISSDIGGYSSVSWYQAHPGKAPKLMIYDVNNRPSGISNRFSGSKSGNTASLAISGLQAEDEADYYCSLYTSINASIVFGGGTKLTVLGQPKAAPSVTLFPPSS

SEQ ID NO: 13 - DNA, 545 bp, Homo sapiens
atgaagcacctgtggttcttccttctgctggtggcggctcccagatgggtcctgtcccagctgcaactgcaggagtcgggcccaggactggtgaagccttcggagaccctgtccctcacctgcactgtctctggtgactccatcagcagtagtacttactactggggctggatccgccagcccccaggaaaggggctggagtggattgcctttatcttttatagcgggagcaccttctacaacccgtccctcaagagtcgagtcaccgtctccgtagacaggtccacgaaccagttctccctgaggctgaagtctgtgaccgccgcagacacgtccagatattactgtgcgagacacccaaaacgtatctcgatttttgaagtggtcaacgcttttgatatctggggccaggggacaatggtcaccgtctcttcagcctccaccaagggcccatcggtcttccccctggcaccctcctccaagagcacctctgggggcacagcggccctgggctgcctggtctgctgacgaggcactgaggactg

SEQ ID NO: 14 - protein, 168 aa, Homo sapiens
MKHLWFFLLLVAAPRWVLSQLQLQESGPGLVKPSETLSLTCTVSGDSISSSTYYWGWIRQPPGKGLEWIAFIFYSGSTFYNPSLKSRVTVSVDRSTNQFSLRLKSVTAADTSRYYCARHPKRISIFEVVNAFDIWGQGTMVTVSSASTKGPSVFPLAPSSKSTSGGTA

SEQ ID NO: 15 - DNA, 465 bp, Homo sapiens
atggcctggactctgctattcctcaccctcctcactcagggcacagggtcctgggcccagtctgccctgactcagcctgcctccgtgtctgggtctcctggacagtcgatcaccatcacctgcactggaatcagcagtgacgttggtgcttataattctgtctcctggtaccagcagtacccaggcaaatcccccaagctcatgatttatgatgtcagtaatcggtcctcaggggtttctaatcgcttctctggctccaagtctgacaacacggcctccctgaccatctctgggctccaggctgaggacgaggcttcttatttctgcagcttatatagaagcagcaccacttccgtggtattcggcggagggaccaagctgaccgtcctacgtcagcccaaggctgccccctcggtcactctgttcccgccctcctctgaggagcttcaagccaacaaggccaca

SEQ ID NO: 16 - protein, 146 aa, Homo sapiens
MAWTLLFLTLLTQGTGSWAQSALTQPASVSGSPGQSITITCTGISSDVGAYNSVSWYQQYPGKSPKLMIYDVSNRSSGVSNRFSGSKSDNTASLTISGLQAEDEASYFCSLYRSSTTSVVFGGGTKLTVLRQPKAAPSVTLFPPSS

SEQ ID NO: 17 - DNA, 432 bp, Oryctolagus sp.
  misc_feature (430)..(430): n is a, c, g, or t
  misc_feature (432)..(432): n is a, c, g, or t
gctagccaccatggagactgggctgcgctggcttctcctggtcgctgtgctcaaaggtgtccagtgtcagtcggtggaggagtccgggggtcgcctggtcacgcctgggacacccctgacactcacctgcatagtctctggaatcgacctcagtagctatgcaatgggctgggtccgccaggctccaggaaaggggctggaatacatcggaatcattagtagcagtggtatcacatactacgcgagctgggcgaaaggccgattcaccatctccaaaacctcgtcgaccacggtgactctgacaatcaccgatctgcaaccttcagacacgggcacctatttctgtgccagagggtctcgttatagtgcttttggtgcttttgatacctggggcccaggcaccctggtcaccgtctcctcagcaagcttnan

SEQ ID NO: 18 - DNA, 444 bp, Oryctolagus sp.
  misc_feature (444)..(444): n is a, c, g, or t
tttggctagccaccatggagactgggctgcgctggcttctcctggtcgctgtgctcaaaggtgtccagtgtcagtcggtggaggagtccgggggtcgcctggtcacgcctgggacacccctgacactcacctgcacagtctctggattctccctcagtagctatgcaatgggctgggtccgccaggctccagggaaggggctggaatggatcggagtcattaataataatggtgacacatactacgcgagctggccgaaaggccgattcaccatctccaaaacctcgaccacggtggatctgaaaatcaccagtccgacaaccgaggacacggccacctatttctgtgccagagatcgtggtaatagttattactttggattggactactttaacttgtggggcccaggcaccctggtcaccgtctcctcagcaagctttatan

SEQ ID NO: 19 - DNA, 385 bp, Oryctolagus sp.
  misc_feature (274)..(274): n is a, c, g, or t
  misc_feature (303)..(303): n is a, c, g, or t
  misc_feature (330)..(330): n is a, c, g, or t
  misc_feature (365)..(365): n is a, c, g, or t
  misc_feature (374)..(374): n is a, c, g, or t
  misc_feature (378)..(378): n is a, c, g, or t
  misc_feature (381)..(381): n is a, c, g, or t
  misc_feature (383)..(385): n is a, c, g, or t
ctctgctgctctggctcccaggtgccagatgtgccttcgaattgacccagactccatcctccgtggaggcagctgtgggaggcacagtcaccatcaagtgccaggccagtcagagtattaatagttggttatcctggtatcagcagaaaccagggcagcctcccaagctcctgatctacaaggcatccaatctggcatctggggtcccatcgcggttcagaggcagtggatctgggacagagttcactctcaccatcagcgacctggagtgtgncgatgctgccacttactactgtcaaagcnattatgctactagtagtgttgattatnatgctttcggcggaaggaccgaggtggtggtcaanactgcggcngtantantnnn

SEQ ID NO: 20 - DNA, 425 bp, Oryctolagus sp.
  misc_feature (416)..(416): n is a, c, g, or t
  misc_feature (425)..(425): n is a, c, g, or t
tgcagctagccaccatggacacgagggcccccatcagctgctggggctcctgctgctctggctcccaggtgccaggtgtgcccttgtgatgacccagactccagcctctgtggaggtagctgtgggaggcacagtcaccatcaagtgccaggccagtcagagcattgatagttggttatcctggtatcagcagaaaccagggcagcgtcccaggctcctgatctattatgcatccaatctggcatctggggtctcatcgcggttcaaaggcagtggatctgggacagaatacactctcaccatcagcggcgtggagtgtgccgatgctgccacttactactgtcaagagggttatagtagtggtaatgttgataatgttttcggcggagggaccgaggtggtggtcaaaactgcgnccgctatan

SEQ ID NO: 21 - DNA, 367 bp, Homo sapiens
gaattccatgcaggtgcagctggtgcagtctggcgccgaagtgaagaaacccggcagcagcgtgaaggtgtcctgcaaggccagcggcctgaccatcagcgacacctacatgcactgggtgcgccaggctccaggccagggactggaatggatgggcagaatcgaccccgccaacggcaacaccaagttcgaccccaagttccagggcagagtgaccatcaccgccgacaccagcacctccaccgcctacatggaactgagcagcctgcggagcgaggacaccgccgtgtactattgtgccagaggcgtgttcggcttcttcgactactggggccagggcaccaccgtgaccgtgtcatctgctagc

SEQ ID NO: 22 - DNA, 405 bp, Homo sapiens
accggtgccaccatgtaccggatgcagctgctgagctgtatcgccctgtctctggccctcgtgacgaattcagccatggacatccagatgacccagagccccagcagcctgtctgccagcgtgggcgacagagtgaccatcacatgcaaggccaccgaggacatctacaaccggctggcctggtatcagcagaagcccggcaaggcccccaagctgctgattagcggagccaccagcctggaaaccggcgtgccaagcagattttccggcagcggctccggcaaggactacaccctgaccatcagctccctgcagcccgaggacttcgccacctactactgccagcagttttggagcgccccctacacctttggcggaggcaccaaggtggaaatcaagcgtacg

SEQ ID NO: 23 - DNA, 357 bp, Mus sp.
atgcaggtgcagctgaaggagtcaggacctggcctggtggcgccctcacagagcctgtccatcacatgcaccgtctcagggttctcattaaccggctatggtgtaaactgggttcgccagcctccaggaaagggtctggagtggctgggaatgatttggggtgatggaaacacagactataattcagctctcaaatccagactgagcatcagcaaggacaactccaagagccaagttttcttaaaaatgaacagtctgcacactgatgacacagccaggtactactgtgccagagagagagattataggcttgactactggggccaaggcaccactctcacagtctcctcagctagc

SEQ ID NO: 24 - DNA, 318 bp, Mus sp.
atggacatccagatgactcagtctccagcctccctttctgcgtctgtgggagaaactgtcaccatcacatgtcgagcaagtgggaatattcacaattatttagcatggtatcagcagaaacagggaaaatctcctcagctcctggtctattatacaacaaccttagcagatggtgtgccatcaaggttcagtggcagtggatcaggaacacaatattctctcaagatcaacagcctgcagcctgaagattttgggagttattactgtcaacatttttggagtactcctcggacgttcggtggaggcaccaagctcgag

SEQ ID NO: 25 - DNA, 357 bp, Mus sp.
atggaggtccagctgcagcagtctggagctgagctgatgaagccaggggcctcagtgaagatatcctgcaaagcttctggctacacattcagtgactactggatagagtgggtaaagcagaggcctggacatggccttgagtggattggagagattttacctggaagtggtagcactaattaccatgagagattcaagggcaaggccacattcactgcagatacatcctccagcacagcctacatgcaactcaacagcctgacatctgaagactctggcgtctattactgcctccatggtaactacgactttgacggctggggccaaggcaccactctcacagtctcctcagctagc

SEQ ID NO: 26 - DNA, 312 bp, Mus sp.
atggatatcgttctcacacagtctccagcaatcatgtctgcatctccaggggagaaggtcaccatgacctgcagtgccagttcaagtgtaaattacatgtactggtaccagcagaagtcaggcacttcccccaaaagatggatttatgacacatccaaactggcttctggagtccctgttcgcttcagtggcagtgggtctgggacctcttactctctcacaatcagcagcatggagactgaagatgctgccacttattactgccaacagtggggtcgtaaccccacgttcggaggggggaccaagctcgag

SEQ ID NO: 27 - DNA, 510 bp, Mus sp.
tggaaggtggtgcacactgctggacagggatccagagttccaggtcactgtcactggctcagggaaatagcccttgaccaggcatcccagggtcaccatggagttagtttgggcagcagatccaggggccagtggatagacagatgggggtgtcgttttggctgaggagactgtgagagtggtgccttggccccagcagtccccgtcccagtttgcacagtaatatgtggctgtgtcctcaggagtcacagaaatcaactgcaggtagcactggttcttggatgtgtctcgagtgatagagattcgacctttgagagatggattgtagtaagtgctaccactgtagcttatgtaccccatatactcaagtttgttccctgggaatttccggatccagctccagtaatcattggtgatggagtcgccagtgacagaacaggtgagggacagagtctgagaaggtttcacgaggctaggtccagactcctgcagctgcacctcgaattccca

SEQ ID NO: 28 - DNA, 342 bp, Mus sp.
ttggtcccccctccgaacgtgtacggccagttgttactctgttgacagaaatacattccaaaatcttcagtctccacactgatgatactgagagtgaaatccgtccctgatccactgccactgaacctggaggggatcccagagatggactgggaagcatacttgatgagaagccttggagactcatgtgatttttgttgataccagtgtaggttgttgctaatactttggctggccctgcaggaaagactgacgctatctcctggagtcacagacagggtgtctggagactgagttagcacaatatcacctctggaggctgaaatccagaaaagcaaaaaa

SEQ ID NO: 29 - DNA, 26 bp, Artificial Sequence
  Template switching primer
  misc_feature (24)..(26): May be ribonucleic acid residues
gcagtggtatcaacgcagagtacggg

SEQ ID NO: 30 - DNA, 24 bp, Artificial Sequence
  Universal primer TS
gcagtggtatcaacgcagagtacg

SEQ ID NO: 31 - DNA, 27 bp, Artificial Sequence
  Universal primer RT
agacagtcctcagtgcctcgtcagcag

SEQ ID NO: 32 - DNA, 13 bp, Artificial Sequence
  Human RT primer HsRT-01
gtcctgaggactg

SEQ ID NO: 33 - DNA, 13 bp, Artificial Sequence
  Human RT primer HsRT-02
tgctctgtgacac

SEQ ID NO: 34 - DNA, 13 bp, Artificial Sequence
  Human RT primer HsRT-03
ggtgtacaggtcc

SEQ ID NO: 35 - DNA, 13 bp, Artificial Sequence
  Human RT primer HsRT-04
cagagagcgtgag

SEQ ID NO: 36 - DNA, 16 bp, Artificial Sequence
  Human RT primer HsRT-05
tcatgtagtagctgtc

SEQ ID NO: 37 - DNA, 14 bp, Artificial Sequence
  Human RT primer HsRT-06
ctcaggactgatgg

SEQ ID NO: 38 - DNA, 15 bp, Artificial Sequence
  Human RT primer HsRT-07
gagtcctgagtactg

SEQ ID NO: 39 - DNA, 16 bp, Artificial Sequence
  Human RT primer HsRT-08
gttgttgctttgtttg

SEQ ID NO: 40 - DNA, 15 bp, Artificial Sequence
  Human RT primer HsRT-09
ttgttgctctgtttg

SEQ ID NO: 41 - DNA, 44 bp, Artificial Sequence
  Long gene-specific primer HsN2U_01
agacagtcctcagtgcctcgtcagcagaccaggcagcccagggc

SEQ ID NO: 42 - DNA, 55 bp, Artificial Sequence
  Long gene-specific primer HsN2U_02
agacagtcctcagtgcctcgtcagcagcagtgtggccttgttggcttgaagctcc

SEQ ID NO: 43 - DNA, 53 bp, Artificial Sequence
  Long gene-specific primer HsN2U_03
agacagtcctcagtgcctcgtcagcagagcaggcacacaacagaggcagttcc

SEQ ID NO: 44 - DNA, 52 bp, Artificial Sequence
  Long gene-specific primer HsN2U_04
agacagtcctcagtgcctcgtcagcaggcccagagtcacggaggtggcattg

SEQ ID NO: 45 - DNA, 54 bp, Artificial Sequence
  Long gene-specific primer HsN2U_05
agacagtcctcagtgcctcgtcagcaggcatgcgacgaccacgttcccatcttg

SEQ ID NO: 46 - DNA, 46 bp, Artificial Sequence
  Long gene-specific primer HsN2U_06
agacagtcctcagtgcctcgtcagcaggcagccaacggccacgctg

SEQ ID NO: 47 - DNA, 57 bp, Artificial Sequence
  Long gene-specific primer HsN2U_07
agacagtcctcagtgcctcgtcagcagatgccaggaccacagggctgttatcctttg

SEQ ID NO: 48 - DNA, 53 bp, Artificial Sequence
  Long gene-specific primer HsN2U_08
agacagtcctcagtgcctcgtcagcagagtgtggccttgttggcttggagctc

SEQ ID NO: 49 - DNA, 51 bp, Artificial Sequence
  Long gene-specific primer HsN2U_09
agacagtcctcagtgcctcgtcagcagaccacgttcccatctggctgggtg

SEQ ID NO: 50 - DNA, 14 bp, Artificial Sequence
  RT mouse primer MmRT_01
acagtcactgagct

SEQ ID NO: 51 - DNA, 15 bp, Artificial Sequence
  RT mouse primer MmRT_02
ctttgacaaggcatc

SEQ ID NO: 52 - DNA, 16 bp, Artificial Sequence
  RT mouse primer MmRT_03
ccacttgacattgatg

SEQ ID NO: 53 - DNA, 15 bp, Artificial Sequence
  RT mouse primer MmRT_04
ctcttctccacagtg

SEQ ID NO: 54 - DNA, 52 bp, Artificial Sequence
  Long gene-specific mouse primer Mmn2_01
agacagtcctcagtgcctcgtcagcagactgcaggagagctgggaaggtgtg

SEQ ID NO: 55 - DNA, 50 bp, Artificial Sequence
  Long gene-specific mouse primer Mmn2_02
agacagtcctcagtgcctcgtcagcaggacagctgggaaggtgtgcacac

SEQ ID NO: 56 - DNA, 53 bp, Artificial Sequence
  Long gene-specific mouse primer Mmn2_03
agacagtcctcagtgcctcgtcagctcaagaagcacacgactgaggcacctcc

SEQ ID NO: 57 - DNA, 50 bp, Artificial Sequence
  Long gene-specific mouse primer Mmn2_04
agacagtcctcagtgcctcgtcagcttgccttccaggccactgtcacacc

SEQ ID NO: 58 - DNA, 53 bp, Artificial Sequence
  Long gene-specific mouse primer Mmn2_05
agacagtcctcagtgcctcgtcagcatccagatgtgtcactgcagccagggac

SEQ ID NO: 59 - DNA, 53 bp, Artificial Sequence
  Long gene-specific mouse primer Mmn2_06
agacagtcctcagtgcctcgtcagcaccttccagtccactgtcaccacacctg

SEQ ID NO: 60 - DNA, 13 bp, Artificial Sequence
  RT rabbit primer OcRT_01
tgaagctctggac

SEQ ID NO: 61 - DNA, 13 bp, Artificial Sequence
  RT rabbit primer OcRT_02
cacactcagaggg

SEQ ID NO: 62 - DNA, 13 bp, Artificial Sequence
  RT rabbit primer OcRT_03
ttccagctcacac

SEQ ID NO: 63 - DNA, 12 bp, Artificial Sequence
  RT rabbit primer OcRT_04
aggaagctgctg

SEQ ID NO: 64 - DNA, 12 bp, Artificial Sequence
  RT rabbit primer OcRT_05
acactgctcagc

SEQ ID NO: 65 - DNA, 14 bp, Artificial Sequence
  RT rabbit primer OcRT_06
tcacattcagaggg

SEQ ID NO: 66 - DNA, 15 bp, Artificial Sequence
  RT rabbit primer OcRT_07
gtcttgtccactttg

SEQ ID NO: 67 - DNA, 14 bp, Artificial Sequence
  RT rabbit primer OcRT_08
ctctgttgctgttg

SEQ ID NO: 68 - DNA, 43 bp, Artificial Sequence
  Long rabbit gene-specific primer Oc-PCR-IgHA1A7-12
agacagtcctcagtgcctcgtcaggatcaggcagccgacgacc

SEQ ID NO: 69 - DNA, 49 bp, Artificial Sequence
  Long rabbit gene-specific primer Oc-PCR-IgKC1
agacagtcctcagtgcctcgtcaggtgggaagatgaggacagtaggtgc

SEQ ID NO: 70 - DNA, 47 bp, Artificial Sequence
  Long rabbit gene-specific primer Oc-PCR-IgKC1KC2
agacagtcctcagtgcctcgtcagagatggtgggaagaggaggacag

SEQ ID NO: 71 - DNA, 51 bp, Artificial Sequence
  Long rabbit gene-specific primer Oc-PCR-IgLC4L5L6
agacagtcctcagtgcctcgtcagccttgttgtccttgagttcctcagagg

SEQ ID NO: 72 - DNA, 44 bp, Artificial Sequence
  Long rabbit gene-specific primer Oc-PCR-IgA2A6
agacagtcctcagtgcctcgtcagcggatcaggcagccgatgac

SEQ ID NO: 73 - DNA, 46 bp, Artificial Sequence
  Long rabbit gene-specific primer Oc-PCR-IgA4A5
agacagtcctcagtgcctcgtcagcaggtcagcgggaagatgatcg

SEQ ID NO: 74 - DNA, 48 bp, Artificial Sequence
  Long rabbit gene-specific primer Oc-PCR-IgLC1C2C3
agacagtcctcagtgcctcgtcagcactgatcagacacaccagggtgg

SEQ ID NO: 75 - DNA, 43 bp, Artificial Sequence
  Long rabbit gene-specific primer Oc-PCR-IgG
agacagtcctcagtgcctcgtcagcaccgtggagctgggtgtg

SEQ ID NO: 76 - DNA, 43 bp, Artificial Sequence
  Long rabbit gene-specific primer Oc-PCR-IgA3A5
agacagtcctcagtgcctcgtcaggatcaggcagccggcgatc

SEQ ID NO: 77 - DNA, 47 bp, Artificial Sequence
  Long rabbit gene-specific primer Oc-PCR-IgM
agacagtcctcagtgcctcgtcagggagacgagcgggtacagagttg

SEQ ID NO: 78 - DNA, 43 bp, Artificial Sequence
  Long rabbit gene-specific primer Oc-PCR-IgE
agacagtcctcagtgcctcgtcagtctgcagcaggaggccaag

SEQ ID NO: 79 - protein, 528 aa, Homo sapiens
MGTSHPAFLVLGCLLTGLSLILCQLSLPSILPNENEKVVQLNSSFSLRCFGESEVSWQYPMSEEESSDVEIRNEENNSGLFVTVLEVSSASAAHTGLYTCYYNHTQTEENELEGRHIYIYVPDPDVAFVPLGMTDYLVIVEDDDSAIIPCRTTDPETPVTLHNSEGVVPASYDSRQGFNGTFTVGPYICEATVKGKKFQTIPFNVYALKATSELDLEMEALKTVYKSGETIVVTCAVFNNEVVDLQWTYPGEVKGKGITMLEEIKVPSIKLVYTLTVPEATVKDSGDYECAARQATREVKEMKKVTISVHEKGFIEIKPTFSQLEAVNLHEVKHFVVEVRAYPPPRISWLKNNLTLIENLTEITTDVEKIQEIRYRSKLKLIRAKEEDSGHYTIVAQNEDAVKSYTFELLTQVPSSILDLVDDHHGSTGGQTVRCTAEGTPLPDIEWMICKDIKKCNNETSWTILANNVSNIITEIHSRDRSTVEGRVTFAKVEETIAVRCLAKNLLGAENRELKLVAPTLRSELTVA

SEQ ID NO: 80 - protein, 528 aa, Mus musculus
MGTSHQVFLVLSCLLTGPGLISCQLLLPSILPNENEKIVQLNSSFSLRCVGESEVSWQHPMSEEDDPNVEIRSEENNSGLFVTVLEVVNASAAHTGWYTCYYNHTQTDESEIEGRHIYIYVPDPDMAFVPLGMTDSLVIVEEDDSAIIPCRTTDPETQVTLHNNGRLVPASYDSRQGFNGTFSVGPYICEATVKGRTFKTSEFNVYALKATSELNLEMDARQTVYKAGETIVVTCAVFNNEVVDLQWTYPGEVRNKGITMLEEIKLPSIKLVYTLTVPKATVKDSGEYECAARQATKEVKEMKRVTISVHEKGFVEIEPTFGQLEAVNLHEVREFVVEVQAYPTPRISWLKDNLTLIENLTEITTDVQKSQETRYQSKLKLIRAKEEDSGHYTIIVQNEDDVKSYTFELSTLVPASILDLVDDHHGSGGGQTVRCTAEGTPLPEIDWMICKHIKKCNNDTSWTVLASNVSNIITELPRRGRSTVEGRVSFAKVEETIAVRCLAKNNLSVVARELKLVAPTLRSELTVA

SEQ ID NO: 81 - protein, 526 aa, Oryctolagus cuniculus
MGPSPPAFLVLVLGWLLAGPSLTRCQLPLPSISPGDSERVVPLNSSFTLRCSGESEVSWQYPVSEDEGPRVDVRSEENNTGYFVAVLEVGSATAAHTGLYTCYYNHTQTEDSDVEGSHVYIYVPDPDVAFVPLGMTDYLVIVEDDDSAIIPCRTTDPETPVTLRNSQGLVPASYDSRHGFNGTFTMGPYVCEATVRGKTVQTIPFNIYALKATSELDLEMEALQTVYKAGETIVVTCAVFNNEVVDLQWTYPGEMKGKGVTMLEEIKVPTLKLVYTLTVPRATVKDSGDYECAARQATEVKEMKKVTIAVHEKGFVEIKPTFNQSEAVNLHEVKHFVVEVRAYPPPRISWLKDSRTLIENLTEITTDVEQVQETRLSSMCNRSAACGKWNFLTSVEQGWQIVQCSAWKAPLAVPATILDLVDDHHPPGEKRVRCTAAGTPPDVEWMICKDIKRCNNETSWTLLANNVSNIVTETHPRGGGAVEGRVTFAKVEETLAVRCLARNPLGTENRELKLVAPTLRSELTVA

SEQ ID NO: 82 - protein, 527 aa, Rattus norvegicus
MGTSQAFLVLSCLLTGPSLIVCQLLLPSILPNENEKIVPLSSSFSLRCFGESEVSWQHPMSEEEDPNVEIRTEENNSSLFVTVLEVVNASAAHTGWYTCYYNHTQTEESEIEGRHIYIYVPDPDMAFVPLGMTDSLVIVEEDDSAIIPCLTTDPDTEVTLHNNGRLVPASYDSRQGFNGTFSVGPYICEATVRGRTFKTSEFNVYALKATSELNLEMDTRQTVYKAGETIVVTCAVFNNEVVDLQWTYPGEVRNKGITMLEEIKLPSIKLVYTLTVPKATVKDSGDYECAARQATKEVKEMKTVTISVHEKGFVQIRPTFGHLETVNLHQVREFVVEVQAYPTPRISWLKDNLTLIENLTEITTDVQRSQETRYQSKLKLIRAKEEDSGHYTIIVQNDDDMKSYTFELSTLVPASILELVDDHHGSGGGQTVRCTAEGTPLPNIEWMICKDIKKCNNDTSWTVLASNVSNIITEFHQRGRSTVEGRVSFAKVEETIAVRCLAKNDLGIGNRELKLVAPSLRSELTVA

SEQ ID NO: 83 - protein, 168 aa, Homo sapiens; identical to SEQ ID NO: 14

SEQ ID NO: 84 - protein, 169 aa, Homo sapiens; identical to SEQ ID NO: 10

SEQ ID NO: 85 - protein, 146 aa, Homo sapiens; identical to SEQ ID NO: 12